European Patent Application EP 4 332 221 A1, published March 6, 2024. Title: THREOSE NUCLEIC ACID ANTISENSE OLIGONUCLEOTIDES AND METHODS THEREOF. Applicant: ROCHE INNOVATION CENTER COPENHAGEN A/S. The sequence listing filed with the application follows.

SEQUENCE LISTING (46 sequences)

SEQ ID NO: 1 - DNA, 16 bp, synthetic construct
  source 1..16: mol_type = other DNA
gagttacttgccaact

SEQ ID NO: 2 - DNA, 20 bp, synthetic construct
  source 1..20: mol_type = other DNA
gccaggctggttatgactca

SEQ ID NO: 3 - DNA, 20 bp, synthetic construct
  source 1..20: mol_type = other DNA
ggcatatgcagataatgttc

SEQ ID NO: 4 - DNA, 20 bp, synthetic construct
  source 1..20: mol_type = other DNA
gggagttacttgccaacttg

SEQ ID NO: 5 - DNA, 20 bp, synthetic construct
  source 1..20: mol_type = other DNA
tgcctttaggattctagaca

SEQ ID NO: 6 - DNA, 20 bp, synthetic construct
  source 1..20: mol_type = other DNA
ccaggctggttatgactcag

SEQ ID NO: 7 - DNA, 20 bp, synthetic construct
  source 1..20: mol_type = other DNA
ttatcaattcaccaaggagc

SEQ ID NO: 8 - DNA, 20 bp, synthetic construct
  source 1..20: mol_type = other DNA
atggaggtatgacatataat

SEQ ID NO: 9 - DNA, 20 bp, synthetic construct
  source 1..20: mol_type = other DNA
gttatgcttattccccaatg

SEQ ID NO: 10 - DNA, 20 bp, synthetic construct
  source 1..20: mol_type = other DNA
ctcagcctttatcactcagc

SEQ ID NO: 11 - DNA, 20 bp, synthetic construct
  source 1..20: mol_type = other DNA
aacaaatttccttagttggc

SEQ ID NO: 12 - DNA, 20 bp, synthetic construct
  source 1..20: mol_type = other DNA
tacaccagtccttttagtag

SEQ ID NO: 13 - DNA, 20 bp, synthetic construct
  source 1..20: mol_type = other DNA
atgctcatcactttatgaag

SEQ ID NO: 14 - DNA, 20 bp, synthetic construct
  source 1..20: mol_type = other DNA
aaaaggcttagcgcccacct

SEQ ID NO: 15 - DNA, 20 bp, synthetic construct
  source 1..20: mol_type = other DNA
aagagaaccacacactacca

SEQ ID NO: 16 - DNA, 20 bp, synthetic construct
  source 1..20: mol_type = other DNA
catctcaacctccgtcatgt

SEQ ID NO: 17 - DNA, 20 bp, synthetic construct
  source 1..20: mol_type = other DNA
aaggtctcatacactcacta

SEQ ID NO: 18 - DNA, 20 bp, synthetic construct
  source 1..20: mol_type = other DNA
gtactatcccatcactgaag

SEQ ID NO: 19 - DNA, 20 bp, synthetic construct
  source 1..20: mol_type = other DNA
gacccctgactttctggaaa

SEQ ID NO: 20 - DNA, 20 bp, synthetic construct
  source 1..20: mol_type = other DNA
cagcggtacactccttctct

SEQ ID NO: 21 - DNA, 20 bp, synthetic construct
  source 1..20: mol_type = other DNA
gccaatatttgcccctcccc

SEQ ID NO: 22 - DNA, 20 bp, synthetic construct
  source 1..20: mol_type = other DNA
tgcatttacttgccaacaga

SEQ ID NO: 23 - DNA, 20 bp, synthetic construct
  source 1..20: mol_type = other DNA
aaagagtaactaccagccat

SEQ ID NO: 24 - DNA, 20 bp, synthetic construct
  source 1..20: mol_type = other DNA
aacaggtcatctattcacaa

SEQ ID NO: 25 - DNA, 20 bp, synthetic construct
  source 1..20: mol_type = other DNA
tgtacattttgcccttagct

SEQ ID NO: 26 - DNA, 20 bp, synthetic construct
  source 1..20: mol_type = other DNA
gccaagcactcatatgcaat

SEQ ID NO: 27 - DNA, 20 bp, synthetic construct
  source 1..20: mol_type = other DNA
gttatgcttattccccaatg

SEQ ID NO: 28 - DNA, 20 bp, synthetic construct
  source 1..20: mol_type = other DNA
gtgtaattaccttttactct

SEQ ID NO: 29 - DNA, 20 bp, synthetic construct
  source 1..20: mol_type = other DNA
ccttcagagattcaatgcta

SEQ ID NO: 30 - DNA, 20 bp, synthetic construct
  source 1..20: mol_type = other DNA
gccaatatttgcccctcccc

SEQ ID NO: 31 - DNA, 20 bp, synthetic construct
  source 1..20: mol_type = other DNA
tgctaaacaaatttccttag

SEQ ID NO: 32 - DNA, 20 bp, synthetic construct
  source 1..20: mol_type = other DNA
aacaaatttccttagttggc

SEQ ID NO: 33 - DNA, 20 bp, synthetic construct
  source 1..20: mol_type = other DNA
tcagtgctattttatccaat

SEQ ID NO: 34 - DNA, 20 bp, synthetic construct
  source 1..20: mol_type = other DNA
tgtacattttgcccttagct

SEQ ID NO: 35 - DNA, 20 bp, synthetic construct
  source 1..20: mol_type = other DNA
ttgctgaaattgtctcaatt

SEQ ID NO: 36 - DNA, 20 bp, synthetic construct
  source 1..20: mol_type = other DNA
ttgaagcataccttaacatc

SEQ ID NO: 37 - DNA, 20 bp, synthetic construct
  source 1..20: mol_type = other DNA
ctccaatacttgtcttagct

SEQ ID NO: 38 - DNA, 20 bp, synthetic construct
  source 1..20: mol_type = other DNA
gccttaaagttacattcgtt

SEQ ID NO: 39 - DNA, 20 bp, synthetic construct
  source 1..20: mol_type = other DNA
aaggtctcatacactcacta

SEQ ID NO: 40 - DNA, 20 bp, synthetic construct
  source 1..20: mol_type = other DNA
gtactatcccatcactgaag

SEQ ID NO: 41 - DNA, 20 bp, synthetic construct
  source 1..20: mol_type = other DNA
atgcaagttaaacttatctg

SEQ ID NO: 42 - DNA, 20 bp, synthetic construct
  source 1..20: mol_type = other DNA
tgcctcttcattgtatttct

SEQ ID NO: 43 - DNA, 20 bp, synthetic construct
  source 1..20: mol_type = other DNA
catcaaggcactgatcactt

SEQ ID NO: 44 - DNA, 20 bp, synthetic construct
  source 1..20: mol_type = other DNA
gccaagcactcatatgcaat

SEQ ID NO: 45 - DNA, 20 bp, synthetic construct
  source 1..20: mol_type = other DNA
gggagttacttgccaacttg

SEQ ID NO: 46 - DNA, 16 bp, synthetic construct
  source 1..16: mol_type = other DNA
gagttacttgccaact